European Patent Specification EP 4 081 659 B1, published October 8, 2025. Title: SIMPLIFIED POLYNUCLEOTIDE SEQUENCE DETECTION METHOD. Applicant: Biofidelity Ltd. The sequence listing filed with the application follows.

SEQUENCE LISTING (35 sequences)

SEQ ID NO: 1 - DNA, 69 bp, Artificial Sequence
  A at position 1 has a 5' phosphate. A, T, G and T (positions 1-4)        are all linked by phosphorothioate bonds.
atgttcgatgagctttgacaatacttgaagctcgcagatataggatgttgcgatagtccaggaggctgc

SEQ ID NO: 2 - DNA, 36 bp, Artificial Sequence
  DNA sequence
tgtcaaagctcatcgaacatcctggactatgtctcc

SEQ ID NO: 3 - DNA, 75 bp, Artificial Sequence
  Part of human EGFR gene
tgctgggcatctgcctcacctccaccgtgcagctcatcacgcagctcatgcccttcggcagcctcctggactatg

SEQ ID NO: 4 - DNA, 75 bp, Artificial Sequence
  Part of human EGFR gene with C797S mutation
tgctgggcatctgcctcacctccaccgtgcagctcatcacgcagctcatgcccttcggctgcctcctggactatg

SEQ ID NO: 5 - DNA, 20 bp, Artificial Sequence
  DNA sequence
tcgcaacatcctatatctgc

SEQ ID NO: 6 - DNA, 20 bp, Artificial Sequence
  DNA Sequence
tgagctttgacaatacttga

SEQ ID NO: 7 - DNA, 90 bp, Artificial Sequence
  WT oligonucleotide
catctgcctcacctccaccgtgcagctcatcacgcagctcatgcccttcggctgcctcctggactatgtccgggaacacaaagacaatat

SEQ ID NO: 8 - DNA, 90 bp, Artificial Sequence
  T790M oligonucleotide
catctgcctcacctccaccgtgcagctcatcatgcagctcatgcccttcggctgcctcctggactatgtccgggaacacaaagacaatat

SEQ ID NO: 9 - DNA, 90 bp, Artificial Sequence
  C797S_2389 oligonucleotide
catctgcctcacctccaccgtgcagctcatcacgcagctcatgcccttcggcagcctcctggactatgtccgggaacacaaagacaatat

SEQ ID NO: 10 - DNA, 78 bp, Artificial Sequence
  T790M probe. 5' phosphate. Phosphorothioate bonds between A, T, G and T at positions 1-4.
atgttcgatgagctttgacaatacttgagcacggcagatataggatgttgcgaagggcatgagctgcatgatgagctg

SEQ ID NO: 11 - DNA, 69 bp, Artificial Sequence; identical to SEQ ID NO: 1
  C797S_2389 probe. 5' phosphate. Phosphorothioate bonds between A, T, G and T at positions 1-4.

SEQ ID NO: 12 - DNA, 36 bp, Artificial Sequence
  T790M splint oligonucleotide.
tgtcaaagctcatcgaacatgcccttcgcaacatct

SEQ ID NO: 13 - DNA, 36 bp, Artificial Sequence
  C797S_2389 splint oligonucleotide.
tgtcaaagctcatcgaacattcctggactatcgcat

SEQ ID NO: 14 - DNA, 70 bp, Artificial Sequence
  Cy5 primer. 3' Qusar670 dye, Quencher between G at position 50 and A at position 51.
acgcctggttaccgagccaggttcgcacatgtaggctcggtaaccaggcgacatcctatatctgccgtgc

SEQ ID NO: 15 - DNA, 58 bp, Artificial Sequence
  TexasRed primer. 5' TexasRed dye. Quencher between G at position 38 and C at position 39.
acgcctggttacaggttcgcacatgtagtaaccaggcgcaacatcctatatctgcgag

SEQ ID NO: 16 - DNA, 20 bp, Artificial Sequence
  Reverse primer.
atgttcgatgagctttgaca

SEQ ID NO: 17 - DNA, 100 bp, Artificial Sequence
  WT oligonucleotide.
cccaaccaagctctcttgaggatcttgaaggaaactgaattcaaaaagatcaaagtgctgggctccggtgcgttcggcacggtgtataaggtaaggtccc

SEQ ID NO: 18 - DNA, 100 bp, Artificial Sequence
  G719X_6239 oligonucleotide.
cccaaccaagctctcttgaggatcttgaaggaaactgaattcaaaaagatcaaagtgctggcctccggtgcgttcggcacggtgtataaggtaaggtccc

SEQ ID NO: 19 - DNA, 100 bp, Artificial Sequence
  G719X_6252 oligonucleotide.
cccaaccaagctctcttgaggatcttgaaggaaactgaattcaaaaagatcaaagtgctgagctccggtgcgttcggcacggtgtataaggtaaggtccc

SEQ ID NO: 20 - DNA, 100 bp, Artificial Sequence
  G719X_6253 oligonucleotide.
cccaaccaagctctcttgaggatcttgaaggaaactgaattcaaaaagatcaaagtgctgtgctccggtgcgttcggcacggtgtataaggtaaggtccc

SEQ ID NO: 21 - DNA, 77 bp, Artificial Sequence
  G719X_6239 probe oligonucleotide. 5' phosphate. Phosphorothioate bonds between A, T, G and T at positions 1-4.
atgttcgatgagctttgacaatacttgacatgcgcagatataggatgttgcgaaacgcaccggaggccagcactttg

SEQ ID NO: 22 - DNA, 77 bp, Artificial Sequence
  G719X_6252 probe oligonucleotide. 5' phosphate. Phosphorothioate bonds between A, T, G and T at positions 1-4.
atgttcgatgagctttgacaatacttgacatgccgagtaatgagagtttcgcaaacgcaccggagctcagcactttg

SEQ ID NO: 23 - DNA, 77 bp, Artificial Sequence
  G719X_6253 probe oligonucleotide. 5' phosphate. Phosphorothioate bonds between A, T, G and T at positions 1-4.
atgttcgatgagctttgacaatacttgacatgcgagcaattaggtagtgtcgtaacgcaccggagcacagcactttg

SEQ ID NO: 24 - DNA, 36 bp, Artificial Sequence
  Splint oligonucleotide.
tgtcaaagctcatcgaacatccggtgcgttcggcaa

SEQ ID NO: 25 - DNA, 59 bp, Artificial Sequence
  Dye primer 1. 5' Cy5 dye, phosphorothioate bond between A at position 1 and C at position 2.
actgaccagctccatgacaatcgctgtcgccatgatcgatcgcaacatcctatatctgc

SEQ ID NO: 26 - DNA, 59 bp, Artificial Sequence
  Dye primer 2. 5' TEX dye, phosphorothioate bond between A at position 1 and C at position 2.
actgaccagctccatgacaatcgctgtcgccatgatcgatgcgaaactctcattactcg

SEQ ID NO: 27 - DNA, 59 bp, Artificial Sequence
  Dye primer 3. 5' TEX dye, phosphorothioate bond between T at position 1 and A at position 2.
tacgaccgactcactccttacagcagtccgcagtatgctacgacactacctaattgctc

SEQ ID NO: 28 - DNA, 39 bp, Artificial Sequence
  Quencher primer 1. 3' Iowa Black RQ quencher.
tcgatcatggcgacagcgattgtcatggagctggtcagt

SEQ ID NO: 29 - DNA, 39 bp, Artificial Sequence
  Quencher primer 2. 3' Iowa Black FQ quencher.
agcatactgcggactgctgtaaggagtgagtcggtcgta

SEQ ID NO: 30 - DNA, 20 bp, Artificial Sequence
  Reverse primer. Phosphorothioate bonds between T, G and A at positions 1-3.
tgagctttgacaatacttga

SEQ ID NO: 31 - DNA, 81 bp, Artificial Sequence
  Wildtype oligo
ctgctgggcatctgcctcacctccaccgtgcagctcatcacgcagctcatgcccttcggctgcctcctggactatgtccgg

SEQ ID NO: 32 - DNA, 81 bp, Artificial Sequence
  Wildtype oligo
ctgctgggcatctgcctcacctccaccgtgcagctcatcatgcagctcatgcccttcggctgcctcctggactatgtccgg

SEQ ID NO: 33 - DNA, 74 bp, Artificial Sequence
  5'phosphate.Phosphorothioate bonds betweeen a,g,c,t at positions 1-4.
agctgcatctgagctttgacaatacttgagcacggcagatataggatgttgcgaagggcatgagctgcatgatg

SEQ ID NO: 34 - DNA, 20 bp, Artificial Sequence
  Phosphorothioate bonds betweeen t,c and g at positions 1-3.
tcgcaacatcctatatctgc

SEQ ID NO: 35 - DNA, 20 bp, Artificial Sequence
atgttgcgaagggcatatgt